European Patent Specification EP 4 274 851 B1, published November 26, 2025. Title: ANTI-GPRC5D MONOCLONAL ANTIBODIES AND USES THEREOF. Applicant: LaNova Medicines Development Co., Ltd. The sequence listing filed with the application follows.

SEQUENCE LISTING (86 sequences)

SEQ ID NO: 1 - protein, 118 aa, Artificial Sequence
  Synthetic
QVQLQQSGAELARPGASVKMSCKASGYTFTTYTMHWVKQRPGQGLEWLGYINPSSGYTNYNQKFKDKATLTAGKSSSTAYMQLSSLTSEDSAVYYCASLRSRGYFDYWGQGTTLTVSS

SEQ ID NO: 2 - protein, 107 aa, Artificial Sequence
  Synthetic
DIVMTQSQTFMSTSVGDRVRITCKASQNVGTAVVWYQQKTGQSPRLLIYSASNRYTGVPDRFTGSGSGTDFTLTISNMQSEDLADFFCQQYSSYPYTFGGGTKLEIK

SEQ ID NO: 3 - protein, 113 aa, Artificial Sequence
  Synthetic
QVQLQQSGAELVRPGTSVKVSCKASGYAFINYLIEWIKQRPGQGLEWIGMINPGSGGTNYNEKFKDKATLTADKSSSTAYMQLSSLTSDDSAVYFCARNWDVWGQGTTLTVSS

SEQ ID NO: 4 - protein, 112 aa, Artificial Sequence
  Synthetic
DVVMTQSPLSLPVSLGDQASVSCRSSQSLVHSTGNTYLHWYLQKPGQSPKLLIYKVSNRFSGVPDRFSGSGSGTDFTLKISRVEAEDLGVYFCSQSTHVPWTFGGGTKLEIK

SEQ ID NO: 5 - protein, 118 aa, Artificial Sequence
  Synthetic
EVQLQQSGPELVKPGASMKLSCKASGYSFTGYTMHWVKQSHGENLEWIGLINPYNGGTNYNQKFKGKATLTVDKSSSTAYMELLSLTSEDSAVYYCSRWGLRRAMDYWGQGTSVTVSS

SEQ ID NO: 6 - protein, 107 aa, Artificial Sequence
  Synthetic
DIVMTQSQKFMSTSVGDRVSVTCKASQNVGSNVAWYQQKPGQSPKALIYSASYRYSGVPDRFTGNGSGTDFTLTISNVQSEDLAEYFCQQYYNSPWTFGGGTKLEIK

SEQ ID NO: 7 - protein, 117 aa, Artificial Sequence
  Synthetic
EVHLVESGGDLVKPGGSLKLSCAASGFTFSSYGMSWVRQTPDKRLEWVATISSGGSYTYYPDSVKGRFTISRDNAKNTLNLQMSSLKSEDTAMYYCARQGGDAMDYWGQGTSVTVSS

SEQ ID NO: 8 - protein, 106 aa, Artificial Sequence
  Synthetic
DIVLTQSPATLSVTPGDSVSLSCRASQSINNNLHWYQQKSHESPRLLIKYASQSISGIPSRFSGSGSGTDFTLSINSVETEDFGMYFCQQSNSRLTFGAGTKLELK

SEQ ID NO: 9 - protein, 124 aa, Artificial Sequence
  Synthetic
EVNLEESGGGLVQPGGSMKLSCVASGFTFSDYWMNWVRQSPEKGLEWVAEIRLKSNNYATHYAESVKGRFTISRDDSKSSVYLQMNNLRAEDTGIYYCTRPLLWFRRYYAMDYWGQGTSVTVSS

SEQ ID NO: 10 - protein, 107 aa, Artificial Sequence
  Synthetic
DIQMTQTTSSLSASLGDRITISCSASQGISNYLNWYQQKPDGTVKLLIYYTSSLHSGVPSRFSGSGSGTDYSLTISNLEPADIATYYCQQYSKLPFTFGSGTKLEIK

SEQ ID NO: 11 - protein, 118 aa, Artificial Sequence
  Synthetic
QVQLQQSGAELARPGASVKMSCKASGYTFTTYTMHWVKQRPGQGLEWIGYINPSSGYTNYNQKFKDKATLTAGKSSSTAYMQLSSLTSEDSAVYYCASLRSRGYFDYWGRGTTLTVSS

SEQ ID NO: 12 - protein, 107 aa, Artificial Sequence
  Synthetic
DIVMTQSQKFLSTSVGDRVSITCKASQNVGTAVAWYQQKPGQSPKLLIYSASNRYTGVPDRFTGSGSGTDFTLTISNMQSEDLAGYFCQQYSSYPYTFGGGTKLEIK

SEQ ID NO: 13 - protein, 122 aa, Artificial Sequence
  Synthetic
EVQLQQSGPELVKPGASVKMSCKASGYTFTRNIMHWVKQKPGQGLEWIGYINPYNAGSKYNEKFKGKATLTSDISSSTAYMELSSLTSEDSAVYYCAREEVYYRYGAWFAYWGHGTLVTVSA

SEQ ID NO: 14 - protein, 111 aa, Artificial Sequence
  Synthetic
DIVLTQSPASLAVSLGQRATISCRASQSVSTSSYSYMHWYQQKPGQPPKLLIKYASNLESGVPARFSGSGSGTDFTLNIHPVEEEDTATYYCQHSWEIPRTFGGGTKLEIK

SEQ ID NO: 15 - protein, 119 aa, Artificial Sequence
  Synthetic
EVQLQQSGPELVKTGASVKISCKASGYSFTGYYIHWVKQSHGKSLEWIGYISCYNGATSFNQKFKGKATFTVDTSSSTAYMQFNSLTSEDSAVYYCARTELRGPWFAYWGQGTLVTVSA

SEQ ID NO: 16 - protein, 106 aa, Artificial Sequence
  Synthetic
QTVLTQSPAIMSASPGEKVTMTCSASSSVSYMNWYQQKSGTSPKRWIYDTSKLASGVPARFSGSGSGTSYSLTISSMEAEDAATYYCQQWSNNPLTFGAGTKLELK

SEQ ID NO: 17 - protein, 113 aa, Artificial Sequence; identical to SEQ ID NO: 3
  Synthetic

SEQ ID NO: 18 - protein, 112 aa, Artificial Sequence; identical to SEQ ID NO: 4
  Synthetic

SEQ ID NO: 19 - protein, 122 aa, Artificial Sequence
  Synthetic
QVHLQQSGAELARPGASVKMSCKASGYTFTTYTMHWVKQRPGQGLEWIGYINPNSAYTNYNQKFKDKATLTADKSSSTAYMQLSSLTSEDSAVYYCARRVLLLRVLDFFDYWGQGTTLTVSS

SEQ ID NO: 20 - protein, 107 aa, Artificial Sequence
  Synthetic
DVQITQSPSYLAASPGETITINCRASKSINKYLTWYQEKPGKTNKLLIYSGSTLQSGIPSRFSGSGSGSDFTLTISSLEPEDFAMYYCQQHNEYPLTFGTGTKLELK

SEQ ID NO: 21 - protein, 118 aa, Artificial Sequence
  Synthetic
EVQLQQSGPELVKPGASMKISCKASGYSFTGYTMNWVKQSHGKNLEWIGLINPYNGGIRYNQKFKGKATLTVDKSSSTAYMELLSLTSEDSAVYYCARWGLRRAMDYWGQGTSVTVSS

SEQ ID NO: 22 - protein, 107 aa, Artificial Sequence
  Synthetic
DIVMTQSQKFMSTSVGDRVSVTCKASQNVGTNVAWYQQKPGQSPKALIYSASYRYSGVPDRFTGSGSGTDFTLTISNVQSEDLAEYFCQQYNSSPWTFGGGTKLEIK

SEQ ID NO: 23 - protein, 118 aa, Artificial Sequence
  Synthetic
EVQLQQSGPELVKPGASMKISCKASGYSFTGYTMNWVKQSHGKNLEWIGLINPYNGGTNYNQKFKGKATLAVDKSSSTAYMDLLSLTSEDSAVYYCSRWGLRRAMDYWGQGTSVTVSS

SEQ ID NO: 24 - protein, 107 aa, Artificial Sequence
  Synthetic
DIVMTQSQKFMSTSVGDRVSVTCKASQNVGSNVAWYQQKPGQSPKALIYSASYRYSGVPDRFTGSGSGTDFTLTISNVQSEDLAEYFCQQYNNSPWTFGGGTKLEIK

SEQ ID NO: 25 - protein, 118 aa, Artificial Sequence
  Synthetic
EVQLQQSGPELVKPGASMKISCKASGYSFTGYTMHWVKQSHGENLEWIGLINPYNGGTNYNQKFKGKATLTVDKSSSTAYMELLSLTSEDSAVYYCSRWGLRRAMDYWGQGTSVTVSS

SEQ ID NO: 26 - protein, 107 aa, Artificial Sequence
  Synthetic
DIVMTQSQKFMSTSIGDRVSVTCKASQNVGSNVAWYQQKPGQSPKALIYSASYRYSGVPDRFTGNGSGTDFTLTISNVQSEDLAEYFCQQYYNSPWTFGGGTKLEIK

SEQ ID NO: 27 - protein, 113 aa, Artificial Sequence
  Synthetic
QVQLQQSGAELVRPGTSVKVSCKASGYAFISYLIEWIKQRPGQGLEWIGMINPGSGGTNYNEKFKDKATLTADKSSSTAYMQLSSLTSDDSAVYFCARNWDVWGQGTTLTVSS

SEQ ID NO: 28 - protein, 112 aa, Artificial Sequence; identical to SEQ ID NO: 4
  Synthetic

SEQ ID NO: 29 - protein, 5 aa, Artificial Sequence
  Synthetic
SYGMS

SEQ ID NO: 30 - protein, 17 aa, Artificial Sequence
  Synthetic
TISSGGSYTYYPDSVKG

SEQ ID NO: 31 - protein, 8 aa, Artificial Sequence
  Synthetic
QGGDAMDY

SEQ ID NO: 32 - protein, 11 aa, Artificial Sequence
  Synthetic
RASQSINNNLH

SEQ ID NO: 33 - protein, 7 aa, Artificial Sequence
  Synthetic
YASQSIS

SEQ ID NO: 34 - protein, 8 aa, Artificial Sequence
  Synthetic
QQSNSRLT

SEQ ID NO: 35 - protein, 117 aa, Artificial Sequence
  Synthetic
EVQLVESGGGLVKPGGSLRLSCAASGFTFSSYGMSWVRQAPGKGLEWVSTISSGGSYTYYPDSVKGRFTISRDNAKNSLYLQMNSLRAEDTAVYYCARQGGDAMDYWGQGTLVTVSS

SEQ ID NO: 36 - protein, 117 aa, Artificial Sequence
  Synthetic
EVQLVESGGGLVKPGGSLRLSCAASGFTFSSYGMSWVRQTPGKGLEWVATISSGGSYTYYPDSVKGRFTISRDNAKNSLYLQMSSLRAEDTAVYYCARQGGDAMDYWGQGTLVTVSS

SEQ ID NO: 37 - protein, 117 aa, Artificial Sequence
  Synthetic
EVHLVESGGGLVKPGGSLRLSCAASGFTFSSYGMSWVRQTPGKRLEWVATISSGGSYTYYPDSVKGRFTISRDNAKNSLNLQMSSLRAEDTAVYYCARQGGDAMDYWGQGTLVTVSS

SEQ ID NO: 38 - protein, 106 aa, Artificial Sequence
  Synthetic
DIQMTQSPSSLSASVGDRVTITCRASQSINNNLHWYQQKPGKAPKLLIYYASQSISGVPSRFSGSGSGTDFTLTISSLQPEDFATYYCQQSNSRLTFGGGTKVEIK

SEQ ID NO: 39 - protein, 106 aa, Artificial Sequence
  Synthetic
DIQMTQSPSSLSASVGDRVTITCRASQSINNNLHWYQQKPGKAPKLLIYYASQSISGIPSRFSGSGSGTDFTLTISSVQPEDFATYFCQQSNSRLTFGGGTKVEIK

SEQ ID NO: 40 - protein, 106 aa, Artificial Sequence
  Synthetic
DIQLTQSPSSLSASVGDRVTITCRASQSINNNLHWYQQKPGKSPKLLIYYASQSISGIPSRFSGSGSGTDFTLTISSVQPEDFATYFCQQSNSRLTFGGGTKLEIK

SEQ ID NO: 41 - protein, 106 aa, Artificial Sequence
  Synthetic
DIVLTQSPSSLSVSVGDRVTLTCRASQSINNNLHWYQQKPGKSPKLLIYYASQSISGIPSRFSGSGSGTDFTLTISSVQPEDFATYFCQQSNSRLTFGGGTKLEIK

SEQ ID NO: 42 - protein, 5 aa, Artificial Sequence
  Synthetic
DYWMN

SEQ ID NO: 43 - protein, 19 aa, Artificial Sequence
  Synthetic
EIRLKSNNYATHYAESVKG

SEQ ID NO: 44 - protein, 13 aa, Artificial Sequence
  Synthetic
PLLWFRRYYAMDY

SEQ ID NO: 45 - protein, 11 aa, Artificial Sequence
  Synthetic
SASQGISNYLN

SEQ ID NO: 46 - protein, 7 aa, Artificial Sequence
  Synthetic
YTSSLHS

SEQ ID NO: 47 - protein, 9 aa, Artificial Sequence
  Synthetic
QQYSKLPFT

SEQ ID NO: 48 - protein, 124 aa, Artificial Sequence
  Synthetic
EVQLVESGGGLVQPGGSLRLSCAASGFTFSDYWMNWVRQAPGKGLEWVAEIRLKSNNYATHYAESVKGRFTISRDNAKNSLYLQMNSLRAEDTAVYYCARPLLWFRRYYAMDYWGQGTLVTVSS

SEQ ID NO: 49 - protein, 124 aa, Artificial Sequence
  Synthetic
EVQLVESGGGLVQPGGSLRLSCAASGFTFSDYWMNWVRQSPGKGLEWVAEIRLKSNNYATHYAESVKGRFTISRDNAKSSLYLQMNSLRAEDTAVYYCTRPLLWFRRYYAMDYWGQGTLVTVSS

SEQ ID NO: 50 - protein, 124 aa, Artificial Sequence
  Synthetic
EVQLVESGGGLVQPGGSLRLSCAASGFTFSDYWMNWVRQSPGKGLEWVAEIRLKSNNYATHYAESVKGRFTISRDDSKSSVYLQMNSLRAEDTAVYYCTRPLLWFRRYYAMDYWGQGTLVTVSS

SEQ ID NO: 51 - protein, 107 aa, Artificial Sequence
  Synthetic
DIQMTQSPSSLSASVGDRVTITCSASQGISNYLNWYQQKPGKAPKLLIYYTSSLHSGVPSRFSGSGSGTDFTLTISSLQPEDFATYYCQQYSKLPFTFGQGTKLEIK

SEQ ID NO: 52 - protein, 107 aa, Artificial Sequence
  Synthetic
DIQMTQSPSSLSASVGDRVTITCSASQGISNYLNWYQQKPGKTVKLLIYYTSSLHSGVPSRFSGSGSGTDYTLTISSLQPEDFATYYCQQYSKLPFTFGQGTKLEIK

SEQ ID NO: 53 - protein, 107 aa, Artificial Sequence
  Synthetic
DIQMTQSPSSLSASVGDRITITCSASQGISNYLNWYQQKPGKTVKLLIYYTSSLHSGVPSRFSGSGSGTDYTLTISSLQPEDFATYYCQQYSKLPFTFGSGTKLEIK

SEQ ID NO: 54 - protein, 5 aa, Artificial Sequence
  Synthetic
GYYIH

SEQ ID NO: 55 - protein, 17 aa, Artificial Sequence
  Synthetic
YISSYNAATSFNQKFKG

SEQ ID NO: 56 - protein, 10 aa, Artificial Sequence
  Synthetic
TELRGPWFAY

SEQ ID NO: 57 - protein, 10 aa, Artificial Sequence
  Synthetic
SASSSVSYMN

SEQ ID NO: 58 - protein, 7 aa, Artificial Sequence
  Synthetic
DTSKLAS

SEQ ID NO: 59 - protein, 9 aa, Artificial Sequence
  Synthetic
QQWSNNPLT

SEQ ID NO: 60 - protein, 17 aa, Artificial Sequence
  Synthetic
YISCYNGATSFNQKFKG

SEQ ID NO: 61 - protein, 119 aa, Artificial Sequence
  Synthetic
QVQLVQSGAEVKKPGASVKVSCKASGYSFTGYYIHWVRQAPGQGLEWMGYISSYNAATSFNQKFKGRVTMTRDTSTSTVYMELSSLRSEDTAVYYCARTELRGPWFAYWGQGTLVTVSS

SEQ ID NO: 62 - protein, 119 aa, Artificial Sequence
  Synthetic
QVQLVQSGAEVKKPGASVKVSCKASGYSFTGYYIHWVRQAPGQGLEWIGYISSYNAATSFNQKFKGRVTFTVDTSTSTVYMELSSLRSEDTAVYYCARTELRGPWFAYWGQGTLVTVSS

SEQ ID NO: 63 - protein, 119 aa, Artificial Sequence
  Synthetic
QVQLVQSGAEVKKPGASVKVSCKASGYSFTGYYIHWVKQAPGQGLEWIGYISSYNAATSFNQKFKGRVTFTVDTSTSTVYMEFSSLRSEDTAVYYCARTELRGPWFAYWGQGTLVTVSS

SEQ ID NO: 64 - protein, 119 aa, Artificial Sequence
  Synthetic
QVQLVQSGAEVKKPGASVKISCKASGYSFTGYYIHWVKQAPGQGLEWIGYISSYNAATSFNQKFKGRATFTVDTSTSTAYMEFSSLRSEDSAVYYCARTELRGPWFAYWGQGTLVTVSS

SEQ ID NO: 65 - protein, 106 aa, Artificial Sequence
  Synthetic
DIQMTQSPSSLSASVGDRVTITCSASSSVSYMNWYQQKPGKAPKLLIYDTSKLASGVPSRFSGSGSGTDFTLTISSLQPEDFATYYCQQWSNNPLTFGQGTKLEIK

SEQ ID NO: 66 - protein, 106 aa, Artificial Sequence
  Synthetic
DTQMTQSPSSLSASVGDRVTITCSASSSVSYMNWYQQKPGKAPKRLIYDTSKLASGVPSRFSGSGSGTDYTLTISSLQPEDFATYYCQQWSNNPLTFGQGTKLEIK

SEQ ID NO: 67 - protein, 106 aa, Artificial Sequence
  Synthetic
DTQLTQSPSSLSASVGDRVTMTCSASSSVSYMNWYQQKPGKAPKRLIYDTSKLASGVPSRFSGSGSGTDYTLTISSMQPEDFATYYCQQWSNNPLTFGQGTKLEIK

SEQ ID NO: 68 - protein, 5 aa, Artificial Sequence
  Synthetic
TYTMH

SEQ ID NO: 69 - protein, 17 aa, Artificial Sequence
  Synthetic
YINPSSGYTNYNQKFKD

SEQ ID NO: 70 - protein, 9 aa, Artificial Sequence
  Synthetic
LRSRGYFDY

SEQ ID NO: 71 - protein, 11 aa, Artificial Sequence
  Synthetic
KASQNVGTAVV

SEQ ID NO: 72 - protein, 7 aa, Artificial Sequence
  Synthetic
SASNRYT

SEQ ID NO: 73 - protein, 9 aa, Artificial Sequence
  Synthetic
QQYSSYPYT

SEQ ID NO: 74 - protein, 118 aa, Artificial Sequence
  Synthetic
QVQLVQSGAEVKKPGASVKVSCKASGYTFTTYTMHWVRQAPGQGLEWMGYINPSSGYTNYNQKFKDRVTMTRDTSTSTVYMELSSLRSEDTAVYYCSRLRSRGYFDYWGQGTLVTVSS

SEQ ID NO: 75 - protein, 118 aa, Artificial Sequence
  Synthetic
QVQLVQSGAEVKKPGASVKVSCKASGYTFTTYTMHWVRQAPGQGLEWLGYINPSSGYTNYNQKFKDRVTMTADTSTSTVYMELSSLRSEDTAVYYCARLRSRGYFDYWGQGTLVTVSS

SEQ ID NO: 76 - protein, 118 aa, Artificial Sequence
  Synthetic
QVQLVQSGAEVAKPGASVKVSCKASGYTFTTYTMHWVKQAPGQGLEWLGYINPSSGYTNYNQKFKDRVTMTADTSTSTVYMELSSLRSEDTAVYYCASLRSRGYFDYWGQGTLVTVSS

SEQ ID NO: 77 - protein, 118 aa, Artificial Sequence
  Synthetic
QVQLVQSGAEVAKPGASVKMSCKASGYTFTTYTMHWVKQAPGQGLEWLGYINPSSGYTNYNQKFKDRVTLTADTSTSTVYMELSSLRSEDTAVYYCASLRSRGYFDYWGQGTLLTVSS

SEQ ID NO: 78 - protein, 118 aa, Artificial Sequence
  Synthetic
QVQLQQSGAEVAKPGASVKMSCKASGYTFTTYTMHWVKQRPGQGLEWLGYINPSSGYTNYNQKFKDRVTLTADKSTSTVYMELSSLRSEDTAVYYCASLRSRGYFDYWGQGTLLTVSS

SEQ ID NO: 79 - protein, 118 aa, Artificial Sequence
  Synthetic
QVQLQQSGAEVAKPGASVKMSCKASGYTFTTYTMHWVKQRPGQGLEWLGYINPSSGYTNYNQKFKDRATLTAGKSTSTVYMELSSLRSEDTAVYYCASLRSRGYFDYWGQGTLLTVSS

SEQ ID NO: 80 - protein, 107 aa, Artificial Sequence
  Synthetic
DIQLTQSPSFLSASVGDRVTITCKASQNVGTAVVWYQQKPGKAPKLLIYSASNRYTGVPSRFSGSGSGTEFTLTISSLQPEDFATYYCQQYSSYPYTFGQGTKLEIK

SEQ ID NO: 81 - protein, 107 aa, Artificial Sequence
  Synthetic
DIQLTQSPSFLSTSVGDRVTITCKASQNVGTAVVWYQQKPGKSPKLLIYSASNRYTGVPSRFSGSGSGTEFTLTISSLQPEDFATFYCQQYSSYPYTFGQGTKLEIK

SEQ ID NO: 82 - protein, 107 aa, Artificial Sequence
  Synthetic
DIQMTQSPSFLSTSVGDRVTITCKASQNVGTAVVWYQQKPGKSPKLLIYSASNRYTGVPSRFSGSGSGTEFTLTISSMQPEDFATFFCQQYSSYPYTFGQGTKLEIK

SEQ ID NO: 83 - protein, 107 aa, Artificial Sequence
  Synthetic
DIVMTQSPSFLSTSVGDRVTITCKASQNVGTAVVWYQQKPGKSPKLLIYSASNRYTGVPDRFSGSGSGTEFTLTISSMQPEDFATFFCQQYSSYPYTFGGGTKLEIK

SEQ ID NO: 84 - protein, 107 aa, Artificial Sequence
  Synthetic
EIVMTQSPATLSVSPGERATLSCKASQNVGTAVVWYQQKPGQAPRLLIYSASNRYTGIPARFSGSGSGTEFTLTISSLQSEDFAVYYCQQYSSYPYTFGQGTKLEIK

SEQ ID NO: 85 - protein, 107 aa, Artificial Sequence
  Synthetic
EIVMTQSPATLSTSPGERATLSCKASQNVGTAVVWYQQKPGQSPRLLIYSASNRYTGIPDRFSGSGSGTEFTLTISSLQSEDFAVFFCQQYSSYPYTFGQGTKLEIK

SEQ ID NO: 86 - protein, 107 aa, Artificial Sequence
  Synthetic
EIVMTQSPATLSTSPGERVTISCKASQNVGTAVVWYQQKPGQSPRLLIYSASNRYTGIPDRFTGSGSGTDFTLTISSMQSEDFAVFFCQQYSSYPYTFGGGTKLEIK